European Patent Specification EP 3 472 208 B9, published October 4, 2023. Title: T CELL RECEPTORS AND USES THEREOF. Applicant: Medigene Immunotherapies GmbH. The sequence listing filed with the application follows.

SEQUENCE LISTING (231 sequences)

SEQ ID NO: 1 - protein, 15 aa, homo sapiens
  MISC_Feature: CDR3 alpha
CAVHSTAQAGTALIF

SEQ ID NO: 2 - protein, 16 aa, homo sapiens
  MISC_feature: CDR3 beta
CASSTHRGQTNYGYTF

SEQ ID NO: 3 - protein, 7 aa, homo sapiens
  MISC_feature: CDR2 alpha
LYSAGEE

SEQ ID NO: 4 - protein, 6 aa, homo sapiens
  MISC_feature: CDR2 beta
YYNGEE

SEQ ID NO: 5 - protein, 6 aa, homo sapiens
  MISC_feature: CDR1 alpha
VSGLRG

SEQ ID NO: 6 - protein, 5 aa, homo sapiens
  MISC_feature: CDR1 beta
SGDLS

SEQ ID NO: 7 - protein, 274 aa, homo sapiens
  MISC_feature: TCR alpha wt full length
MEKMLECAFIVLWLQLGWLSGEDQVTQSPEALRLQEGESSSLNCSYTVSGLRGLFWYRQDPGKGPEFLFTLYSAGEEKEKERLKATLTKKESFLHITAPKPEDSATYLCAVHSTAQAGTALIFGKGTTLSVSSNIQNPDPAVYQLRDSKSSDKSVCLFTDFDSQTNVSQSKDSDVYITDKTVLDMRSMDFKSNSAVAWSNKSDFACANAFNNSIIPEDTFFPSPESSCDVKLVEKSFETDTNLNFQNLSVIGFRILLLKVAGFNLLMTLRLWSS

SEQ ID NO: 8 - protein, 311 aa, homo sapiens
  MISC_feature: TCR beta wt full length
MGFRLLCCVAFCLLGAGPVDSGVTQTPKHLITATGQRVTLRCSPRSGDLSVYWYQQSLDQGLQFLIQYYNGEERAKGNILERFSAQQFPDLHSELNLSSLELGDSALYFCASSTHRGQTNYGYTFGSGTRLTVVEDLNKVFPPEVAVFEPSEAEISHTQKATLVCLATGFFPDHVELSWWVNGKEVHSGVSTDPQPLKEQPALNDSRYCLSSRLRVSATFWQNPRNHFRCQVQFYGLSENDEWTQDRAKPVTQIVSAEAWGRADCGFTSVSYQQGVLSATILYEILLGKATLYAVLVSALVLMAMVKRKDF

SEQ ID NO: 9 - protein, 274 aa, artificial; identical to SEQ ID NO: 7
  TCR alpha full length humC

SEQ ID NO: 10 - protein, 311 aa, artificial; identical to SEQ ID NO: 8
  TCR beta  humC full length

SEQ ID NO: 11 - protein, 274 aa, artificial
  TCR alpha mmcys full length
MEKMLECAFIVLWLQLGWLSGEDQVTQSPEALRLQEGESSSLNCSYTVSGLRGLFWYRQDPGKGPEFLFTLYSAGEEKEKERLKATLTKKESFLHITAPKPEDSATYLCAVHSTAQAGTALIFGKGTTLSVSSNIQNPDPAVYQLRDSKSSDKSVCLFTDFDSQTNVSQSKDSDVYITDKCVLDMRSMDFKSNSAVAWSNKSDFACANAFNNSIIPEDTFFPSSDVPCDVKLVEKSFETDTNLNFQNLSVIGFRILLLKVAGFNLLMTLRLWSS

SEQ ID NO: 12 - protein, 311 aa, artificial
  TCR beta mmcys full length
MGFRLLCCVAFCLLGAGPVDSGVTQTPKHLITATGQRVTLRCSPRSGDLSVYWYQQSLDQGLQFLIQYYNGEERAKGNILERFSAQQFPDLHSELNLSSLELGDSALYFCASSTHRGQTNYGYTFGSGTRLTVVEDLNKVFPPEVAVFEPSKAEIAHTQKATLVCLATGFFPDHVELSWWVNGKEVHSGVCTDPQPLKEQPALNDSRYCLSSRLRVSATFWQNPRNHFRCQVQFYGLSENDEWTQDRAKPVTQIVSAEAWGRADCGITSASYHQGVLSATILYEILLGKATLYAVLVSALVLMAMVKRKDF

SEQ ID NO: 13 - protein, 270 aa, artificial
  TCR alpha murC full length
MEKMLECAFIVLWLQLGWLSGEDQVTQSPEALRLQEGESSSLNCSYTVSGLRGLFWYRQDPGKGPEFLFTLYSAGEEKEKERLKATLTKKESFLHITAPKPEDSATYLCAVHSTAQAGTALIFGKGTTLSVSSNIQNPEPAVYQLKDPRSQDSTLCLFTDFDSQINVPKTMESGTFITDKTVLDMKAMDSKSNGAIAWSNQTSFTCQDIFKETNATYPSSDVPCDATLTEKSFETDMNLNFQNLSVMGLRILLLKVAGFNLLMTLRLWSS

SEQ ID NO: 14 - protein, 307 aa, artificial
  TCR beta murC full length
MGFRLLCCVAFCLLGAGPVDSGVTQTPKHLITATGQRVTLRCSPRSGDLSVYWYQQSLDQGLQFLIQYYNGEERAKGNILERFSAQQFPDLHSELNLSSLELGDSALYFCASSTHRGQTNYGYTFGSGTRLTVVEDLRNVTPPKVTLFEPSKAEIANKQKATLVCLARGFFPDHVELSWWVNGKEVHSGVSTDPQAYKESNYSYCLSSRLRVSATFWHNPRNHFRCQVQFHGLSEEDKWPEGSPKPVTQNISAEAWGRADCGITSASYHQGVLSATILYEILLGKATLYAVLVSGLVLMAMVKKKNS

SEQ ID NO: 15 - protein, 134 aa, homo sapiens
  MISC_feature: TCR alpha variable
MEKMLECAFIVLWLQLGWLSGEDQVTQSPEALRLQEGESSSLNCSYTVSGLRGLFWYRQDPGKGPEFLFTLYSAGEEKEKERLKATLTKKESFLHITAPKPEDSATYLCAVHSTAQAGTALIFGKGTTLSVSSN

SEQ ID NO: 16 - protein, 134 aa, artificial
  TCR beta variable
  MISC_feature: TCR beta variable
MGFRLLCCVAFCLLGAGPVDSGVTQTPKHLITATGQRVTLRCSPRSGDLSVYWYQQSLDQGLQFLIQYYNGEERAKGNILERFSAQQFPDLHSELNLSSLELGDSALYFCASSTHRGQTNYGYTFGSGTRLTVV

SEQ ID NO: 17 - protein, 140 aa, homo sapiens
  MISC_FEATURE: TCR alpha wt constant
IQNPDPAVYQLRDSKSSDKSVCLFTDFDSQTNVSQSKDSDVYITDKTVLDMRSMDFKSNSAVAWSNKSDFACANAFNNSIIPEDTFFPSPESSCDVKLVEKSFETDTNLNFQNLSVIGFRILLLKVAGFNLLMTLRLWSS

SEQ ID NO: 18 - protein, 177 aa, homo sapiens
  MISC_FEATURE: TCR beta wt constant
EDLNKVFPPEVAVFEPSEAEISHTQKATLVCLATGFFPDHVELSWWVNGKEVHSGVSTDPQPLKEQPALNDSRYCLSSRLRVSATFWQNPRNHFRCQVQFYGLSENDEWTQDRAKPVTQIVSAEAWGRADCGFTSVSYQQGVLSATILYEILLGKATLYAVLVSALVLMAMVKRKDF

SEQ ID NO: 19 - protein, 140 aa, artificial
  TCR alpha minimal murinized constant
  MISC_feature: TCR alpha mmcys constant
IQNPDPAVYQLRDSKSSDKSVCLFTDFDSQTNVSQSKDSDVYITDKCVLDMRSMDFKSNSAVAWSNKSDFACANAFNNSIIPEDTFFPSSDVPCDVKLVEKSFETDTNLNFQNLSVIGFRILLLKVAGFNLLMTLRLWSS

SEQ ID NO: 20 - protein, 177 aa, artificial
  TCR beta minimally murinized C
  MISC_feature: TCR beta mmcys constant
EDLNKVFPPEVAVFEPSKAEIAHTQKATLVCLATGFFPDHVELSWWVNGKEVHSGVCTDPQPLKEQPALNDSRYCLSSRLRVSATFWQNPRNHFRCQVQFYGLSENDEWTQDRAKPVTQIVSAEAWGRADCGITSASYHQGVLSATILYEILLGKATLYAVLVSALVLMAMVKRKDF

SEQ ID NO: 21 - protein, 136 aa, mus musculus
  MISC_FEATURE: TCR alpha murC constant
IQNPEPAVYQLKDPRSQDSTLCLFTDFDSQINVPKTMESGTFITDKTVLDMKAMDSKSNGAIAWSNQTSFTCQDIFKETNATYPSSDVPCDATLTEKSFETDMNLNFQNLSVMGLRILLLKVAGFNLLMTLRLWSS

SEQ ID NO: 22 - protein, 173 aa, mus musculus
  MISC_feature: TCR beta murC constant
EDLRNVTPPKVTLFEPSKAEIANKQKATLVCLARGFFPDHVELSWWVNGKEVHSGVSTDPQAYKESNYSYCLSSRLRVSATFWHNPRNHFRCQVQFHGLSEEDKWPEGSPKPVTQNISAEAWGRADCGITSASYHQGVLSATILYEILLGKATLYAVLVSGLVLMAMVKKKNS

SEQ ID NO: 23 - DNA, 825 bp, homo sapiens
  MISC_feature: TCR alpha wt
atggagaaaatgttggagtgtgcattcatagtcttgtggcttcagcttggctggttgagtggagaagaccaggtgacgcagagtcccgaggccctgagactccaggagggagagagtagcagtcttaactgcagttacacagtcagcggtttaagagggctgttctggtataggcaagatcctgggaaaggccctgaattcctcttcaccctgtattcagctggggaagaaaaggagaaagaaaggctaaaagccacattaacaaagaaggaaagctttctgcacatcacagcccctaaacctgaagactcagccacttatctctgtgctgtgcactccacagcccaggcaggaactgctctgatctttgggaagggaaccaccttatcagtgagttccaatatccagaaccctgaccctgccgtgtaccagctgagagactctaaatccagtgacaagtctgtctgcctattcaccgattttgattctcaaacaaatgtgtcacaaagtaaggattctgatgtgtatatcacagacaaaactgtgctagacatgaggtctatggacttcaagagcaacagtgctgtggcctggagcaacaaatctgactttgcatgtgcaaacgccttcaacaacagcattattccagaagacaccttcttccccagcccagaaagttcctgtgatgtcaagctggtcgagaaaagctttgaaacagatacgaacctaaactttcaaaacctgtcagtgattgggttccgaatcctcctcctgaaagtggccgggtttaatctgctcatgacgctgcggctgtggtccagctga

SEQ ID NO: 24 - DNA, 936 bp, homo sapiens
  MISC_feature: TCR beta wt
atgggcttcaggctcctctgctgtgtggccttttgtctcctgggagcaggcccagtggattctggagtcacacaaaccccaaagcacctgatcacagcaactggacagcgagtgacgctgagatgctcccctaggtctggagacctctctgtgtactggtaccaacagagcctggaccagggcctccagttcctcattcagtattataatggagaagagagagcaaaaggaaacattcttgaacgattctccgcacaacagttccctgacttgcactctgaactaaacctgagctctctggagctgggggactcagctttgtatttctgtgccagcagcacacacagggggcagactaactatggctacaccttcggttcggggaccaggttaaccgttgtagaggacctgaacaaggtgttcccacccgaggtcgctgtgtttgagccatcagaagcagagatctcccacacccaaaaggccacactggtgtgcctggccacaggcttcttccccgaccacgtggagctgagctggtgggtgaatgggaaggaggtgcacagtggggtcagcacggacccgcagcccctcaaggagcagcccgccctcaatgactccagatactgcctgagcagccgcctgagggtctcggccaccttctggcagaacccccgcaaccacttccgctgtcaagtccagttctacgggctctcggagaatgacgagtggacccaggatagggccaaacccgtcacccagatcgtcagcgccgaggcctggggtagagcagactgtggctttacctcggtgtcctaccagcaaggggtcctgtctgccaccatcctctatgagatcctgctagggaaggccaccctgtatgctgtgctggtcagcgcccttgtgttgatggccatggtcaagagaaaggatttctga

SEQ ID NO: 25 - DNA, 825 bp, artificial
  TCR alpha humC codon-optimized
atggaaaagatgctggaatgcgccttcatcgtgctgtggctgcagctgggatggctgagcggagaggaccaagtgacccagtctcccgaggccctgagactgcaggaaggcgagagcagcagcctgaactgcagctacaccgtgtccggcctgagaggcctgttctggtacagacaggaccccggcaagggccccgagttcctgttcacactgtactctgccggcgaggaaaaagagaaagagcggctgaaggccaccctgaccaagaaagagagcttcctgcacatcaccgcccccaagcctgaggacagcgccacatatctgtgcgccgtgcactctacagcccaggccggaaccgccctgatctttggcaagggcaccaccctgagcgtgtccagcaacatccagaatccggaccctgccgtgtaccagctgagagactctaaatccagtgacaagtctgtctgcctattcaccgattttgattctcaaacaaatgtgtcacaaagtaaggattctgatgtgtatatcacagacaaaactgtgctagacatgaggtctatggacttcaagagcaacagtgctgtggcctggagcaacaaatctgactttgcatgtgcaaacgccttcaacaacagcattattccagaagacaccttcttccccagcccagaaagttcctgtgatgtcaagctggtcgagaaaagctttgaaacagatacgaacctaaactttcaaaacctgtcagtgattgggttccgaatcctcctcctgaaagtggccgggtttaatctgctcatgacgctgcggctgtggtccagctga

SEQ ID NO: 26 - DNA, 936 bp, artificial
  TCR beta humC codon-optimized
atgggctttagactgctgtgctgcgtggccttctgcctgctgggagctggccctgtggatagcggcgtgacccagacacccaagcacctgatcacagccaccggccagcgcgtgaccctgagatgttctcctagaagcggcgacctgagcgtgtactggtatcagcagagcctggaccagggcctgcagttcctgatccagtactacaacggcgaggaacgggccaagggcaacatcctggaacggttcagcgcccagcagttccccgatctgcacagcgagctgaacctgagcagcctggaactgggcgacagcgccctgtacttctgtgccagcagcacccacagaggccagaccaactacggctacaccttcggcagcggcaccagactgaccgtggtggaggacctgaacaaagtgttcccacccgaggtcgctgtgtttgagccatcagaagcagagatctcccacacccaaaaggccacactggtgtgcctggccacaggcttcttccccgaccacgtggagctgagctggtgggtgaatgggaaggaggtgcacagtggggtcagcacggacccgcagcccctcaaggagcagcccgccctcaatgactccagatactgcctgagcagccgcctgagggtctcggccaccttctggcagaacccccgcaaccacttccgctgtcaagtccagttctacgggctctcggagaatgacgagtggacccaggatagggccaaacccgtcacccagatcgtcagcgccgaggcctggggtagagcagactgtggctttacctcggtgtcctaccagcaaggggtcctgtctgccaccatcctctatgagatcctgctagggaaggccaccctgtatgctgtgctggtcagcgcccttgtgttgatggccatggtcaagagaaaggatttctga

SEQ ID NO: 27 - DNA, 825 bp, artificial
  TCR alpha mmcys codon-optimized
atggaaaagatgctggaatgcgccttcatcgtgctgtggctgcagctgggatggctgagcggagaggaccaagtgacccagtctcccgaggccctgagactgcaggaaggcgagagcagcagcctgaattgcagctacaccgtgtccggcctgcggggcctgttctggtatagacaggaccctggcaagggccccgagttcctgtttaccctgtactctgccggcgaagagaaagaaaaagagcggctgaaggccacactgaccaagaaagagagcttcctgcacatcaccgcccccaagcctgaggacagcgccacatatctgtgcgccgtgcactctacagcccaggccggaaccgccctgatcttcggcaagggcacaaccctgtccgtgtccagcaacatccagaaccccgaccccgccgtgtaccagctgagagacagcaagagcagcgacaagagcgtgtgcctgttcaccgacttcgacagccagacaaacgtgtcccagagcaaggacagcgacgtgtacatcaccgataagtgcgtgctggacatgcggagcatggacttcaagagcaacagcgccgtggcctggtccaacaagagcgatttcgcctgcgccaacgccttcaacaacagcattatccccgaggacacattcttccccagctccgacgtgccctgcgacgtgaagctggtggaaaagagcttcgagacagacaccaacctgaacttccagaatctgagcgtgatcggcttcagaatcctgctgctgaaggtggccggcttcaatctgctgatgaccctgcggctgtggtccagctga

SEQ ID NO: 28 - DNA, 935 bp, artificial
  TCR beta mmcys codon-optimized
atgggcttccggctgctgtgttgcgtggccttctgtctgctgggagccggccctgtggatagcggcgtgacacagacacccaagcacctgatcaccgccaccggccagcgcgtgacactgagatgtagccctagaagcggcgacctgagcgtgtactggtatcagcagagcctggaccagggcctgcagttcctgatccagtactacaacggcgaggaacgggccaagggcaacatcctggaacggttcagcgcccagcagttccccgatctgcacagcgagctgaacctgagcagcctggaactgggcgacagcgccctgtacttctgtgccagcagcacccacagaggccagaccaactacggctacaccttcggcagcggcaccagactgaccgtggtggaagatctgaacaaggtgttccccccagaggtggccgtgttcgagcctagcaaggccgagatcgcccacacccagaaagccaccctcgtgtgtctggccaccggctttttccccgaccacgtggaactgtcttggtgggtcaacggcaaagaggtgcactccggcgtgtgcaccgatccccagcctctgaaagaacagcccgccctgaacgacagccggtactgcctgtccagcagactgagagtgtccgccaccttctggcagaacccccggaaccacttcagatgccaggtgcagttctacggcctgagcgagaacgacgagtggacccaggacagagccaagcccgtgacccagatcgtgtctgccgaagcctggggcagagccgattgtggcatcaccagcgccagctaccatcagggcgtgctgagcgccaccatcctgtacgagatcctgctgggcaaggccaccctgtacgccgtgctggtgtctgccctggtgctgatggccatggtcaagcggaaggactttga

SEQ ID NO: 29 - DNA, 813 bp, artificial
  TCR alpha murC codon-optimized
atggaaaagatgctggaatgcgccttcatcgtgctgtggctgcagctgggatggctgagcggagaggaccaagtgacccagtctcccgaggccctgagactgcaggaaggcgagagcagcagcctgaactgcagctacaccgtgtccggcctgagaggcctgttctggtacagacaggaccccggcaagggccccgagttcctgttcacactgtactctgccggcgaggaaaaagagaaagagcggctgaaggccaccctgaccaagaaagagagcttcctgcacatcaccgcccccaagcctgaggacagcgccacatatctgtgcgccgtgcactctacagcccaggccggaaccgccctgatctttggcaagggcaccaccctgagcgtgtccagcaacatccagaaccccgagcccgccgtgtaccagctgaaggaccctagaagccaggacagcaccctgtgcctgttcaccgacttcgacagccagatcaacgtgcccaagaccatggaaagcggcaccttcatcaccgacaagacagtgctggacatgaaggccatggacagcaagagcaacggcgccattgcctggtccaaccagaccagcttcacatgccaggacatcttcaaagagacaaacgccacctaccccagcagcgacgtgccctgcgacgccaccctgaccgagaagagcttcgagacagacatgaacctgaatttccagaacctgagcgtgatgggcctgcggatcctgctgctgaaggtggccggcttcaacctgctgatgaccctgcggctgtggagcagctga

SEQ ID NO: 30 - DNA, 924 bp, artificial
  TCR beta murC codon-optimized
atgggctttagactgctgtgctgcgtggccttctgcctgctgggagctggccctgtggatagcggcgtgacccagacacccaagcacctgatcacagccaccggccagcgcgtgaccctgagatgttctcctagaagcggcgacctgagcgtgtactggtatcagcagagcctggaccagggcctgcagttcctgatccagtactacaacggcgaggaacgggccaagggcaacatcctggaacggttcagcgcccagcagttccccgatctgcacagcgagctgaacctgagcagcctggaactgggcgacagcgccctgtacttctgtgccagcagcacccacagaggccagaccaactacggctacaccttcggcagcggcaccagactgaccgtggtggaagatctgcggaacgtgaccccccccaaggtgaccctgttcgagcccagcaaggccgagatcgccaacaagcagaaagccaccctggtctgcctggccaggggcttcttccccgaccacgtggagctgtcttggtgggtgaacggcaaagaggtgcacagcggagtcagtaccgacccccaggcctacaaagagagcaactacagctactgcctgagcagcaggctgagagtgagcgccaccttctggcacaacccccggaaccacttccggtgccaggtgcagttccacggcctgagcgaagaggacaagtggcctgagggcagccccaagcccgtgacccagaacatcagcgccgaggcctggggcagagccgactgcggcatcaccagcgccagctaccaccagggcgtgctgtccgccaccatcctgtacgagatcctgctgggcaaggccaccctgtacgccgtgctggtgtccggcctggtgctgatggccatggtgaagaagaagaacagctga

SEQ ID NO: 31 - protein, 9 aa, artificial
  MINIMAL RECOGNITION SEQUENCE
  MISC_FEATURE (1)..(1): X can be selected from any amino acid
  MISC_FEATURE (3)..(3): X can be selected from any amino acid
  MISC_FEATURE (7)..(7): X can be selected from any amino acid
XLXGLDXLL

SEQ ID NO: 32 - protein, 9 aa, homo sapiens
VLDGLDVLL

SEQ ID NO: 33 - protein, 509 aa, homo sapiens
MERRRLWGSIQSRYISMSVWTSPRRLVELAGQSLLKDEALAIAALELLPRELFPPLFMAAFDGRHSQTLKAMVQAWPFTCLPLGVLMKGQHLHLETFKAVLDGLDVLLAQEVRPRRWKLQVLDLRKNSHQDFWTVWSGNRASLYSFPEPEAAQPMTKKRKVDGLSTEAEQPFIPVEVLVDLFLKEGACDELFSYLIEKVKRKKNVLRLCCKKLKIFAMPMQDIKMILKMVQLDSIEDLEVTCTWKLPTLAKFSPYLGQMINLRRLLLSHIHASSYISPEKEEQYIAQFTSQFLSLQCLQALYVDSLFFLRGRLDQLLRHVMNPLETLSITNCRLSEGDVMHLSQSPSVSQLSVLSLSGVMLTDVSPEPLQALLERASATLQDLVFDECGITDDQLLALLPSLSHCSQLTTLSFYGNSISISALQSLLQHLIGLSNLTHVLYPVPLESYEDIHGTLHLERLAYLHARLRELLCELGRPSMVWLSANPCPHCGDRTFYDPEPILCPCFMPN

SEQ ID NO: 34 - protein, 6 aa, Homo sapiens
TSGFYG

SEQ ID NO: 35 - protein, 6 aa, Homo sapiens
TSGFNG

SEQ ID NO: 36 - protein, 6 aa, Homo sapiens
VSNAYN

SEQ ID NO: 37 - protein, 6 aa, Homo sapiens
VSGNPY

SEQ ID NO: 38 - protein, 7 aa, Homo sapiens
NIATNDY

SEQ ID NO: 39 - protein, 6 aa, Homo sapiens
DSSSTY

SEQ ID NO: 40 - protein, 6 aa, Homo sapiens
NYSPAY

SEQ ID NO: 41 - protein, 6 aa, Homo sapiens
VSRFNN

SEQ ID NO: 42 - protein, 6 aa, Homo sapiens
YGGTVN

SEQ ID NO: 43 - protein, 6 aa, Homo sapiens
SSYSPS

SEQ ID NO: 44 - protein, 6 aa, Homo sapiens
YGATPY

SEQ ID NO: 45 - protein, 6 aa, Homo sapiens
SSVPPY

SEQ ID NO: 46 - protein, 6 aa, Homo sapiens
SSVSVY

SEQ ID NO: 47 - protein, 6 aa, Homo sapiens
TTQYPS

SEQ ID NO: 48 - protein, 6 aa, Homo sapiens
ATGYPS

SEQ ID NO: 49 - protein, 6 aa, Homo sapiens
VSPFSN

SEQ ID NO: 50 - protein, 6 aa, Homo sapiens
ERTLFN

SEQ ID NO: 51 - protein, 6 aa, Homo sapiens
NSASQS

SEQ ID NO: 52 - protein, 6 aa, Homo sapiens
DRGSQS

SEQ ID NO: 53 - protein, 6 aa, Homo sapiens
NSAFQY

SEQ ID NO: 54 - protein, 6 aa, Homo sapiens
DSASNY

SEQ ID NO: 55 - protein, 6 aa, Homo sapiens
NSASDY

SEQ ID NO: 56 - protein, 7 aa, Homo sapiens
TSDPSYG

SEQ ID NO: 57 - protein, 6 aa, Homo sapiens
YSGSPE

SEQ ID NO: 58 - protein, 5 aa, Homo sapiens
TSINN

SEQ ID NO: 59 - protein, 6 aa, Homo sapiens
SSYSTF

SEQ ID NO: 60 - protein, 7 aa, Homo sapiens
TRDTTYY

SEQ ID NO: 61 - protein, 6 aa, Homo sapiens
VSGLRG

SEQ ID NO: 62 - protein, 6 aa, Homo sapiens
DSAIYN

SEQ ID NO: 63 - protein, 5 aa, Homo sapiens
DSVNN

SEQ ID NO: 64 - protein, 6 aa, Homo sapiens
NTAFDY

SEQ ID NO: 65 - protein, 6 aa, Homo sapiens
SSNFYA

SEQ ID NO: 66 - protein, 5 aa, Homo sapiens
TTLSN

SEQ ID NO: 67 - protein, 7 aa, Homo sapiens
TISGNEY

SEQ ID NO: 68 - protein, 7 aa, Homo sapiens
TISGTDY

SEQ ID NO: 69 - protein, 5 aa, Homo sapiens
SVFSS

SEQ ID NO: 70 - protein, 6 aa, Homo sapiens
NSMFDY

SEQ ID NO: 71 - protein, 5 aa, Homo sapiens
KALYS

SEQ ID NO: 72 - protein, 5 aa, Homo sapiens
KTLYG

SEQ ID NO: 73 - protein, 5 aa, Homo sapiens
SIFNT

SEQ ID NO: 74 - protein, 6 aa, Homo sapiens
VTNFRS

SEQ ID NO: 75 - protein, 7 aa, Homo sapiens
TSENNYY

SEQ ID NO: 76 - protein, 7 aa, Homo sapiens
TSESDYY

SEQ ID NO: 77 - protein, 5 aa, Homo sapiens
TTSDR

SEQ ID NO: 78 - protein, 6 aa, Homo sapiens
STGYPT

SEQ ID NO: 79 - protein, 5 aa, Homo sapiens
VGISA

SEQ ID NO: 80 - protein, 5 aa, Homo sapiens
SNHLY

SEQ ID NO: 81 - protein, 5 aa, Homo sapiens
LGHDT

SEQ ID NO: 82 - protein, 5 aa, Homo sapiens
MGHRA

SEQ ID NO: 83 - protein, 5 aa, Homo sapiens
LGHNA

SEQ ID NO: 84 - protein, 5 aa, Homo sapiens
LGHNA

SEQ ID NO: 85 - protein, 5 aa, Homo sapiens
SGHRS

SEQ ID NO: 86 - protein, 5 aa, homo sapiens
SGHNT

SEQ ID NO: 87 - protein, 5 aa, Homo sapiens
SGHKS

SEQ ID NO: 88 - protein, 5 aa, Homo sapiens
SGHDT

SEQ ID NO: 89 - protein, 5 aa, Homo sapiens
SGHTS

SEQ ID NO: 90 - protein, 5 aa, homo sapiens
MNHNS

SEQ ID NO: 91 - protein, 5 aa, Homo sapiens
MNHEY

SEQ ID NO: 92 - protein, 5 aa, Homo sapiens
MNHEY

SEQ ID NO: 93 - protein, 5 aa, homo sapiens
MRHNA

SEQ ID NO: 94 - protein, 5 aa, Homo sapiens
MNHEY

SEQ ID NO: 95 - protein, 5 aa, Homo sapiens
MNHNY

SEQ ID NO: 96 - protein, 5 aa, Homo sapiens
MNHGY

SEQ ID NO: 97 - protein, 5 aa, Homo sapiens
MNHGY

SEQ ID NO: 98 - protein, 5 aa, Homo sapiens
SGHTA

SEQ ID NO: 99 - protein, 5 aa, Homo sapiens
SGHTA

SEQ ID NO: 100 - protein, 5 aa, Homo sapiens
SGHVT

SEQ ID NO: 101 - protein, 5 aa, Homo sapiens
SGHVS

SEQ ID NO: 102 - protein, 5 aa, Homo sapiens
SSHAT

SEQ ID NO: 103 - protein, 5 aa, Homo sapiens
SGHVS

SEQ ID NO: 104 - protein, 5 aa, Homo sapiens
SEHNR

SEQ ID NO: 105 - protein, 5 aa, Homo sapiens
SGDLS

SEQ ID NO: 106 - protein, 5 aa, Homo sapiens
WNHNN

SEQ ID NO: 107 - protein, 5 aa, Homo sapiens
WSHSY

SEQ ID NO: 108 - protein, 5 aa, Homo sapiens
ENHRY

SEQ ID NO: 109 - protein, 5 aa, Homo sapiens
SGHAT

SEQ ID NO: 110 - protein, 5 aa, Homo sapiens
SGHAT

SEQ ID NO: 111 - protein, 5 aa, Homo sapiens
SGHNT

SEQ ID NO: 112 - protein, 5 aa, Homo sapiens
SGHND

SEQ ID NO: 113 - protein, 5 aa, Homo sapiens
FGHNF

SEQ ID NO: 114 - protein, 5 aa, Homo sapiens
SGHNS

SEQ ID NO: 115 - protein, 5 aa, Homo sapiens
SGHDY

SEQ ID NO: 116 - protein, 5 aa, Homo sapiens
LGHNT

SEQ ID NO: 117 - protein, 5 aa, Homo sapiens
PRHDT

SEQ ID NO: 118 - protein, 5 aa, Homo sapiens
SGHDN

SEQ ID NO: 119 - protein, 5 aa, Homo sapiens
LNHNV

SEQ ID NO: 120 - protein, 5 aa, Homo sapiens
KGHSY

SEQ ID NO: 121 - protein, 5 aa, Homo sapiens
KGHSH

SEQ ID NO: 122 - protein, 5 aa, Homo sapiens
LNHDA

SEQ ID NO: 123 - protein, 6 aa, Homo sapiens
DFQATT

SEQ ID NO: 124 - protein, 5 aa, homo sapiens
KGHDR

SEQ ID NO: 125 - protein, 5 aa, Homo sapiens
MGHDK

SEQ ID NO: 126 - protein, 5 aa, Homo sapiens
MNHEY

SEQ ID NO: 127 - protein, 5 aa, Homo sapiens
MDHEN

SEQ ID NO: 128 - protein, 5 aa, Homo sapiens
SQVTM

SEQ ID NO: 129 - protein, 6 aa, Homo sapiens
GTSNPN

SEQ ID NO: 130 - protein, 6 aa, Homo sapiens
NALDGL

SEQ ID NO: 131 - protein, 6 aa, Homo sapiens
NVLDGL

SEQ ID NO: 132 - protein, 4 aa, Homo sapiens
GSKP

SEQ ID NO: 133 - protein, 8 aa, Homo sapiens
YITGDNLV

SEQ ID NO: 134 - protein, 5 aa, Homo sapiens
GYKTK

SEQ ID NO: 135 - protein, 7 aa, homo sapiens
IFSNMDM

SEQ ID NO: 136 - protein, 7 aa, Homo sapiens
IRENEKE

SEQ ID NO: 137 - protein, 7 aa, Homo sapiens
MYSAGYE

SEQ ID NO: 138 - protein, 8 aa, Homo sapiens
YFSGDPLV

SEQ ID NO: 139 - protein, 8 aa, Homo sapiens
YTSAATLV

SEQ ID NO: 140 - protein, 8 aa, Homo sapiens
YFSGDTLV

SEQ ID NO: 141 - protein, 8 aa, Homo sapiens
YTSAATLV

SEQ ID NO: 142 - protein, 8 aa, Homo sapiens
YLSGSTLV

SEQ ID NO: 143 - protein, 7 aa, Homo sapiens
AMKANDK

SEQ ID NO: 144 - protein, 7 aa, Homo sapiens
ATKADDK

SEQ ID NO: 145 - protein, 7 aa, Homo sapiens
MTFSENT

SEQ ID NO: 146 - protein, 7 aa, Homo sapiens
IQSSQKE

SEQ ID NO: 147 - protein, 6 aa, Homo sapiens
VYSSGN

SEQ ID NO: 148 - protein, 6 aa, Homo sapiens
IYSNGD

SEQ ID NO: 149 - protein, 6 aa, Homo sapiens
TYSSGN

SEQ ID NO: 150 - protein, 7 aa, Homo sapiens
IRSNVGE

SEQ ID NO: 151 - protein, 7 aa, Homo sapiens
IRSNMDK

SEQ ID NO: 152 - protein, 8 aa, Homo sapiens
QGSYDQQN

SEQ ID NO: 153 - protein, 4 aa, Homo sapiens
HISR

SEQ ID NO: 154 - protein, 7 aa, Homo sapiens
IRSNERE

SEQ ID NO: 155 - protein, 6 aa, Homo sapiens
SSENQE

SEQ ID NO: 156 - protein, 8 aa, Homo sapiens
RNSFDEQN

SEQ ID NO: 157 - protein, 7 aa, Homo sapiens
LYSAGEE

SEQ ID NO: 158 - protein, 7 aa, Homo sapiens
IQSSQRE

SEQ ID NO: 159 - protein, 5 aa, Homo sapiens
IPSGT

SEQ ID NO: 160 - protein, 7 aa, homo sapiens
IRPDVSE

SEQ ID NO: 161 - protein, 7 aa, Homo sapiens
MTLNGDE

SEQ ID NO: 162 - protein, 7 aa, Homo sapiens
LVKSGEV

SEQ ID NO: 163 - protein, 5 aa, Homo sapiens
GLKNN

SEQ ID NO: 164 - protein, 5 aa, homo sapiens
GLTSN

SEQ ID NO: 165 - protein, 7 aa, Homo sapiens
VVTGGEV

SEQ ID NO: 166 - protein, 7 aa, Homo sapiens
ISSIKDK

SEQ ID NO: 167 - protein, 7 aa, Homo sapiens
LLKGGEQ

SEQ ID NO: 168 - protein, 7 aa, Homo sapiens
LQKGGEE

SEQ ID NO: 169 - protein, 7 aa, Homo sapiens
LYKAGEL

SEQ ID NO: 170 - protein, 7 aa, Homo sapiens
LTSSGIE

SEQ ID NO: 171 - protein, 8 aa, homo sapiens
QEAYKQQN

SEQ ID NO: 172 - protein, 8 aa, Homo sapiens
QEAYKQQN

SEQ ID NO: 173 - protein, 7 aa, Homo sapiens
LLSNGAV

SEQ ID NO: 174 - protein, 4 aa, Homo sapiens
ETME

SEQ ID NO: 175 - protein, 5 aa, Homo sapiens
LSSGK

SEQ ID NO: 176 - protein, 6 aa, Homo sapiens
FYNNEI

SEQ ID NO: 177 - protein, 6 aa, Homo sapiens
YNNKEL

SEQ ID NO: 178 - protein, 6 aa, Homo sapiens
YSYEKL

SEQ ID NO: 179 - protein, 6 aa, Homo sapiens
YNFKEQ

SEQ ID NO: 180 - protein, 6 aa, homo sapiens
YSLEER

SEQ ID NO: 181 - protein, 6 aa, Homo sapiens
YFSETQ

SEQ ID NO: 182 - protein, 6 aa, Homo sapiens
YYREEE

SEQ ID NO: 183 - protein, 6 aa, Homo sapiens
YYEKEE

SEQ ID NO: 184 - protein, 6 aa, Homo sapiens
YYEEEE

SEQ ID NO: 185 - protein, 6 aa, Homo sapiens
YDEGEE

SEQ ID NO: 186 - protein, 6 aa, Homo sapiens
SASEGT

SEQ ID NO: 187 - protein, 6 aa, Homo sapiens
SVGEGT

SEQ ID NO: 188 - protein, 6 aa, Homo sapiens
SVGEGT

SEQ ID NO: 189 - protein, 6 aa, Homo sapiens
SNTAGT

SEQ ID NO: 190 - protein, 6 aa, Homo sapiens
SVGAGI

SEQ ID NO: 191 - protein, 6 aa, Homo sapiens
SVGAGI

SEQ ID NO: 192 - protein, 6 aa, Homo sapiens
SAAAGT

SEQ ID NO: 193 - protein, 6 aa, Homo sapiens
SVAAGI

SEQ ID NO: 194 - protein, 6 aa, Homo sapiens
FQGNSA

SEQ ID NO: 195 - protein, 6 aa, Homo sapiens
FQGTGA

SEQ ID NO: 196 - protein, 6 aa, Homo sapiens
SQSDAQ

SEQ ID NO: 197 - protein, 6 aa, Homo sapiens
FNYEAQ

SEQ ID NO: 198 - protein, 6 aa, Homo sapiens
FNYEAQ

SEQ ID NO: 199 - protein, 6 aa, homo sapiens
FQNEAQ

SEQ ID NO: 200 - protein, 6 aa, Homo sapiens
FQNEAQ

SEQ ID NO: 201 - protein, 6 aa, Homo sapiens
YYNGEE

SEQ ID NO: 202 - protein, 6 aa, Homo sapiens
SYGVQD

SEQ ID NO: 203 - protein, 6 aa, Homo sapiens
SAAADI

SEQ ID NO: 204 - protein, 6 aa, Homo sapiens
SYGVKD

SEQ ID NO: 205 - protein, 6 aa, Homo sapiens
FQDESV

SEQ ID NO: 206 - protein, 6 aa, Homo sapiens
FQNNGV

SEQ ID NO: 207 - protein, 6 aa, Homo sapiens
YENEEA

SEQ ID NO: 208 - protein, 6 aa, Homo sapiens
FCSWTL

SEQ ID NO: 209 - protein, 5 aa, Homo sapiens
FRSSI

SEQ ID NO: 210 - protein, 6 aa, Homo sapiens
FNNNVP

SEQ ID NO: 211 - protein, 6 aa, Homo sapiens
FNNNVP

SEQ ID NO: 212 - protein, 6 aa, Homo sapiens
FRNRAP

SEQ ID NO: 213 - protein, 6 aa, homo sapiens
FYEKMQ

SEQ ID NO: 214 - protein, 6 aa, Homo sapiens
FVKESK

SEQ ID NO: 215 - protein, 6 aa, Homo sapiens
FVKESK

SEQ ID NO: 216 - protein, 6 aa, Homo sapiens
FQNENV

SEQ ID NO: 217 - protein, 6 aa, Homo sapiens
LQKENI

SEQ ID NO: 218 - protein, 6 aa, Homo sapiens
SQIVND

SEQ ID NO: 219 - protein, 7 aa, Homo sapiens
SNEGSKA

SEQ ID NO: 220 - protein, 6 aa, Homo sapiens
SFDVKD

SEQ ID NO: 221 - protein, 6 aa, Homo sapiens
SYGVNS

SEQ ID NO: 222 - protein, 6 aa, Homo sapiens
SMNVEV

SEQ ID NO: 223 - protein, 6 aa, Homo sapiens
SYDVKM

SEQ ID NO: 224 - protein, 5 aa, Homo sapiens
SVGIG

SEQ ID NO: 225 - protein, 5 aa, Artificial
  Linker
GGGGS

SEQ ID NO: 226 - protein, 18 aa, artificial
  linker
KESGSVSSEQLAQFRSLD

SEQ ID NO: 227 - protein, 14 aa, artificial
  linker
EGKSSGSGSESKST

SEQ ID NO: 228 - protein, 12 aa, artificial
  linker
GSAGSAAGSGEF

SEQ ID NO: 229 - protein, 9 aa, artificial
  SLL peptide
SLLQHLIGL

SEQ ID NO: 230 - protein, 10 aa, artificial
  ALY peptide
ALYVDSLFFL

SEQ ID NO: 231 - protein, 10 aa, artificial
  ELA peptide
ELAGIGILTV